European Patent Specification EP 3 082 469 B1, published September 6, 2023. Title: RNAPII NUCLEIC ACID MOLECULES. Applicant: Dow AgroSciences LLC Narva, Ken Arora, Kanika Rangasamy, Murugesan Veeramani, Balajii Gandra, Premchand Worden, Sarah E Li, Huarong Vilcinskas, Andreas Knorr, Eileen. The sequence listing filed with the application follows.

SEQUENCE LISTING (82 sequences)

SEQ ID NO: 1 - DNA, 3745 bp, Diabrotica virgerifera
cggactgtcaaagtcaaatgtcaaagcgtcaaaactaaaatttgctagcgtcaaaactaaaatcaaaatcggcaaacatctgcacgaaaatagagttgtgcttctatatttattttgtaattttgagtaccataatatactaagatgtatgatcaagaagatgatcaatttgacgatgaagatacagaagaaatcagtggagaactctggcaggaagcctgctggattgttattaatgcctactttgatgaaaaaggtttggtacggcagcagttggatagttttgatgaattcattcaaatgtctgtacagaggatcgttgaagattccccacagatagatctacaagcagaagcgcagcatacatctggggaaatcgaaaccccacctcgatatttgctgaagtttgaacagatctatctttcaaaacctacccattgggagaaagacggtgccccatctcctatgatgcctaatgaagctagattaagaaatttgacttattctgctcctctttatgtagatataacaaaaacaattgtgaaagaaggagaggatcctatagaaactcaacatcagaaaacttttataggtaaaattcccattatgttgaggtcaacatactgtctgctcagtggattaacagatcgtgatttaacagaattaaacgagtgtcccttagatcctggcggatatttcataattaacggttctgaaaaagtattaattgctcaagagaagatggcaactaacacagtatatgtattttcaatgaaagacggaaaatatgcgtacaaatctgaaataagatcttgtcttgagcacagctctcggccaacatcaactctgtgggtaaatatgatggctcgtggtggccaggccatcaaaaaagctgctattggtcaacgtattatagctattcttccatacatcaaacaagagatccctataatgatagttttcagagctttagggtttgtagcagacagagatattctagaacacattatttacgatttcgacgatccagaattgatggaaatggtaaaaccttcgttagatgaagctttcgtaattcaggaacagaatattgctttgaatttcatcggagcgagaggtgccaggccgggagtaactaaagaaaagcgtgtgaaatatgctagagaaattttacaaaaggaaatgttgcctcatgttggtgtatccgatttttgtgagactaaaaaagcttattttcttggatatatggtacatcgacttttgctggctgcactcggacgtcgagagttagatgacagagatcactacggaaataagagactcgatttggctggaccattattggctttcctcttcagagggcttttcaagaacctaatgaaagaagttcgtatgtatgcccagaagtttatcgatagaggcaaagatttcaatctggatctggccatcaaaaccaaactaataacggacggtctgaggtattctctcgctactggaaactggggtgaccagaaaaaagcccatcaagcaagagctggcgtgtcccaggtattgaatcgtctaactttcgcatcgacgttgtcacatttaaggcgtgtcaattctccaattggacgagacggtaaactagccaagcctcgacagttgcataatacgttgtggggaatgatttgccctgctgaaactccagaaggtgctgctgtaggacttgtaaaaaatcttgctctgatggcttatatttccgtcggttcccaaccatcgccaattttggagttcttggaggagtggtccatggaaaacttggaagaaatagcgccatctgcaattgctaacgctaccaaaatctttgtgaatggttgttgggtgggaattcacagagaccctgaacaacttatggcgacactgcgtaaacttcgacgtcaaatggacatcatcgtatcagaagtatcgatgattcgagatattcgtgacagagaaataagaatttacacagacgccggaagaatctgtagacctttgttaatcgtcgaaaatggccagttgctattgaagaaaagacatattgatatgttaaaagaaagagaatataataattatggttggcaggtactggtcgcgtctggtgtggtggagtacatagacaccttagaagaagaaaccgtaatgattgccatgaaccccgaagatttacgccaagacaaagaatgcgcttattgtacaacatacactcattgtgaaattcatccagccatgattttaggagtttgcgcttccatcattccgttcccagatcacaaccagagtcccagaaacacctatcaaagtgctatgggtaaacaagccatgggtgtctatatcacaaacttccacgttagaatggacacactggcccacgtcctgtactatccacataaacctctggtaacgacaagatctatggagtatcttagattcagagagttaccggctggaatcaatagtatcgttgcgattgcttgttatacaggatacaatcaggaagattctgttatcttgaatgcttctgcagtagaaagaggatttttcagatctgtgttttaccggtcttataaagacgccgaatccaaacgtataggagaccaggaagaacaattcgaaaaaccgacaagacagacgtgccagggcatgaggaatgccctttacgataaattagacgacgacggactgatatctccaggtattcgtgtgtctggagacgatgtagttataggaaaaactatgacgctaccagaaacagatgacgagttggatggaactacaaaacggtactccaagagagacgcatcaacatttttgcgtaacagtgaaactggagttgttgatcaagtgatgttaacgctaaattcagaaggatataagttttgtaagataagggtgagatctgtgaggataccacaaattggagacaagttcgcgtctaggcacggacaaaagggaacgtgcggtatacaataccgtcaagaggatatgatttttagtgctgaaggtattactccagacattatcatcaatcctcacgctatcccctcccgtatgacgattggtcacttgatcgagtgcatccaaggtaaggtatcatccaataaaggagaaatcggtgatgctacacctttcaacgatgccgtcaacgtacagaaaatctccactttgttacaagaatatggttatcaactcagaggcaacgaagtaatgtacaacggccacactggacgtaagataaatgctcagattttcttaggacctacttactatcaaagattgaagcacatggtggacgataagatccattcaagagctagaggaccgttgcagattctcgtcagacagcctatggagggtcgtgcaagagacggtggtctacgtttcggtgagatggaacgagattgtcaaatttcacacggtgctgcacaattcttaagagagaggctgtttgaagtttctgatccttatagaatccatatttgcaacttctgtggtttgatagctatcgccaatttgcgtaacaacacctttgaatgtaagggttgcaaaaataagacgcagatatcgcaagttagactgccttatgctgcgaaattactgttccaagagctaatgtcgatgaatatagcgccgagacttatggtactgtagtgttttaagtaataaaataaatgtccttatttaagagtattttatattgaaataaacaataaaattataaaaa

SEQ ID NO: 2 - protein, 1175 aa, Diabrotica virgerifera
MYDQEDDQFDDEDTEEISGELWQEACWIVINAYFDEKGLVRQQLDSFDEFIQMSVQRIVEDSPQIDLQAEAQHTSGEIETPPRYLLKFEQIYLSKPTHWEKDGAPSPMMPNEARLRNLTYSAPLYVDITKTIVKEGEDPIETQHQKTFIGKIPIMLRSTYCLLSGLTDRDLTELNECPLDPGGYFIINGSEKVLIAQEKMATNTVYVFSMKDGKYAYKSEIRSCLEHSSRPTSTLWVNMMARGGQAIKKAAIGQRIIAILPYIKQEIPIMIVFRALGFVADRDILEHIIYDFDDPELMEMVKPSLDEAFVIQEQNIALNFIGARGARPGVTKEKRVKYAREILQKEMLPHVGVSDFCETKKAYFLGYMVHRLLLAALGRRELDDRDHYGNKRLDLAGPLLAFLFRGLFKNLMKEVRMYAQKFIDRGKDFNLDLAIKTKLITDGLRYSLATGNWGDQKKAHQARAGVSQVLNRLTFASTLSHLRRVNSPIGRDGKLAKPRQLHNTLWGMICPAETPEGAAVGLVKNLALMAYISVGSQPSPILEFLEEWSMENLEEIAPSAIANATKIFVNGCWVGIHRDPEQLMATLRKLRRQMDIIVSEVSMIRDIRDREIRIYTDAGRICRPLLIVENGQLLLKKRHIDMLKEREYNNYGWQVLVASGVVEYIDTLEEETVMIAMNPEDLRQDKECAYCTTYTHCEIHPAMILGVCASIIPFPDHNQSPRNTYQSAMGKQAMGVYITNFHVRMDTLAHVLYYPHKPLVTTRSMEYLRFRELPAGINSIVAIACYTGYNQEDSVILNASAVERGFFRSVFYRSYKDAESKRIGDQEEQFEKPTRQTCQGMRNALYDKLDDDGLISPGIRVSGDDVVIGKTMTLPETDDELDGTTKRYSKRDASTFLRNSETGVVDQVMLTLNSEGYKFCKIRVRSVRIPQIGDKFASRHGQKGTCGIQYRQEDMIFSAEGITPDIIINPHAIPSRMTIGHLIECIQGKVSSNKGEIGDATPFNDAVNVQKISTLLQEYGYQLRGNEVMYNGHTGRKINAQIFLGPTYYQRLKHMVDDKIHSRARGPLQILVRQPMEGRARDGGLRFGEMERDCQISHGAAQFLRERLFEVSDPYRIHICNFCGLIAIANLRNNTFECKGCKNKTQISQVRLPYAAKLLFQELMSMNIAPRLMVL

SEQ ID NO: 3 - DNA, 468 bp, Diabrotica virgerifera
cctacccattgggagaaagacggtgccccatctcctatgatgcctaatgaagctagattaagaaatttgacttattctgctcctctttatgtagatataacaaaaacaattgtgaaagaaggagaggatcctatagaaactcaacatcagaaaacttttataggtaaaattcccattatgttgaggtcaacatactgtctgctcagtggattaacagatcgtgatttaacagaattaaacgagtgtcccttagatcctggcggatatttcataattaacggttctgaaaaagtattaattgctcaagagaagatggcaactaacacagtatatgtattttcaatgaaagacggaaaatatgcgtacaaatctgaaataagatcttgtcttgagcacagctctcggccaacatcaactctgtgggtaaatatgatggctcgtggtggccaggccatcaaaaaagctgct

SEQ ID NO: 4 - DNA, 180 bp, Diabrotica virgerifera
aaataagagactcgatttggctggaccattattggctttcctcttcagagggcttttcaagaacctaatgaaagaagttcgtatgtatgcccagaagtttatcgatagaggcaaagatttcaatctggatctggccatcaaaaccaaactaataacggacggtctgaggtattctctcgc

SEQ ID NO: 5 - DNA, 161 bp, Diabrotica virgerifera
ttctgcagtagaaagaggatttttcagatctgtgttttaccggtcttataaagacgccgaatccaaacgtataggagaccaggaagaacaattcgaaaaaccgacaagacagacgtgccagggcatgaggaatgccctttacgataaattagacgacgacg

SEQ ID NO: 6 - DNA, 24 bp, Artificial Sequence
  T7 phage promoter
ttaatacgactcactatagggaga

SEQ ID NO: 7 - DNA, 503 bp, Artificial Sequence
  YFP coding region segment
caccatgggctccagcggcgccctgctgttccacggcaagatcccctacgtggtggagatggagggcaatgtggatggccacaccttcagcatccgcggcaagggctacggcgatgccagcgtgggcaaggtggatgcccagttcatctgcaccaccggcgatgtgcccgtgccctggagcaccctggtgaccaccctgacctacggcgcccagtgcttcgccaagtacggccccgagctgaaggatttctacaagagctgcatgcccgatggctacgtgcaggagcgcaccatcaccttcgagggcgatggcaatttcaagacccgcgccgaggtgaccttcgagaatggcagcgtgtacaatcgcgtgaagctgaatggccagggcttcaagaaggatggccacgtgctgggcaagaatctggagttcaatttcaccccccactgcctgtacatctggggcgatcaggccaatcacggcctgaagagcgccttcaagatct

SEQ ID NO: 8 - DNA, 45 bp, Artificial Sequence
  RNAPreg1-F1T7 PCR Primer Oligonucleotide
ttaatacgactcactatagggagacctacccattgggagaaagac

SEQ ID NO: 9 - DNA, 43 bp, Artificial Sequence
  RNAPreg1R1T7 PCR Primer Oligonucleotide
ttaatacgactcactatagggagaagcagcttttttgatggcc

SEQ ID NO: 10 - DNA, 47 bp, Artificial Sequence
  RNAPreg 2 F1T7 PCR Primer Oligonucleotide
ttaatacgactcactatagggagaaaataagagactcgatttggctg

SEQ ID NO: 11 - DNA, 44 bp, Artificial Sequence
  RNAPreg2 R1T7 PCR Primer Oligonucleotide
ttaatacgactcactatagggagagcgagagaatacctcagacc

SEQ ID NO: 12 - DNA, 49 bp, Artificial Sequence
  RNAPreg 3 -F1T7 PCR Primer Oligonucleotide
ttaatacgactcactatagggagattctgcagtagaaagaggatttttc

SEQ ID NO: 13 - DNA, 49 bp, Artificial Sequence
  RNAPreg 3 R1T7 PCR Primer Oligonucleotide
ttaatacgactcactatagggagagtcgtcgtctaatttatcgtaaagg

SEQ ID NO: 14 - DNA, 47 bp, Artificial Sequence
  YFP-F_T7 PCR Primer Oligonucleotide
ttaatacgactcactatagggagacaccatgggctccagcggcgccc

SEQ ID NO: 15 - DNA, 47 bp, Artificial Sequence
  YFP-R_T7 PCR Primer Oligonucleotide
ttaatacgactcactatagggagaagatcttgaaggcgctcttcagg

SEQ ID NO: 16 - DNA, 585 bp, Artificial Sequence
  RNAPII-140 hairpin-RNA-forming sequence v1
aaataagagactcgatttggctggaccattattggctttcctcttcagagggcttttcaagaacctaatgaaagaagttcgtatgtatgcccagaagtttatcgatagaggcaaagatttcaatctggatctggccatcaaaaccaaactaataacggacggtctgaggtattctctcgcgactagtaccggttgggaaaggtatgtttctgcttctacctttgatatatatataataattatcactaattagtagtaatatagtatttcaagtatttttttcaaaataaaagaatgtagtatatagctattgcttttctgtagtttataagtgtgtatattttaatttataacttttctaatatatgaccaaaacatggtgatgtgcaggttgatccgcggttagcgagagaatacctcagaccgtccgttattagtttggttttgatggccagatccagattgaaatctttgcctctatcgataaacttctgggcatacatacgaacttctttcattaggttcttgaaaagccctctgaagaggaaagccaataatggtccagccaaatcgagtctcttattt

SEQ ID NO: 17 - DNA, 545 bp, Artificial Sequence
  RNAPII-140 hairpin-RNA-forming sequence v2
ttctgcagtagaaagaggatttttcagatctgtgttttaccggtcttataaagacgccgaatccaaacgtataggagaccaggaagaacaattcgaaaaaccgacaagacagacgtgccagggcatgaggaatgccctttacgataaattagacgacgacgactagtaccggttgggaaaggtatgtttctgcttctacctttgatatatatataataattatcactaattagtagtaatatagtatttcaagtatttttttcaaaataaaagaatgtagtatatagctattgcttttctgtagtttataagtgtgtatattttaatttataacttttctaatatatgaccaaaacatggtgatgtgcaggttgatccgcggttagtcgtcgtctaatttatcgtaaagggcattcctcatgccctggcacgtctgtcttgtcggtttttcgaattgttcttcctggtctcctatacgtttggattcggcgtctttataagaccggtaaaacacagatctgaaaaatcctctttctactgcagaa

SEQ ID NO: 18 - DNA, 471 bp, Artificial Sequence
  YFP hairpin-RNA-forming sequence v2
atgtcatctggagcacttctctttcatgggaagattccttacgttgtggagatggaagggaatgttgatggccacacctttagcatacgtgggaaaggctacggagatgcctcagtgggaaaggactagtaccggttgggaaaggtatgtttctgcttctacctttgatatatatataataattatcactaattagtagtaatatagtatttcaagtatttttttcaaaataaaagaatgtagtatatagctattgcttttctgtagtttataagtgtgtatattttaatttataacttttctaatatatgaccaaaacatggtgatgtgcaggttgatccgcggttactttcccactgaggcatctccgtagcctttcccacgtatgctaaaggtgtggccatcaacattcccttccatctccacaacgtaaggaatcttcccatgaaagagaagtgctccagatgacat

SEQ ID NO: 19 - DNA, 225 bp, Solanum tuberosum
gactagtaccggttgggaaaggtatgtttctgcttctacctttgatatatatataataattatcactaattagtagtaatatagtatttcaagtatttttttcaaaataaaagaatgtagtatatagctattgcttttctgtagtttataagtgtgtatattttaatttataacttttctaatatatgaccaaaacatggtgatgtgcaggttgatccgcggtta

SEQ ID NO: 20 - DNA, 702 bp, Artificial Sequence
  Plant-optimized yellow fluorescent protein coding region
atgtcatctggagcacttctctttcatgggaagattccttacgttgtggagatggaagggaatgttgatggccacacctttagcatacgtgggaaaggctacggagatgcctcagtgggaaaggttgatgcacagttcatctgcacaactggtgatgttcctgtgccttggagcacacttgtcaccactctcacctatggagcacagtgctttgccaagtatggtccagagttgaaggacttctacaagtcctgtatgccagatggctatgtgcaagagcgcacaatcacctttgaaggagatggcaacttcaagactagggctgaagtcacctttgagaatgggtctgtctacaatagggtcaaactcaatggtcaaggcttcaagaaagatggtcatgtgttgggaaagaacttggagttcaacttcactccccactgcctctacatctggggtgaccaagccaaccacggtctcaagtcagccttcaagatctgtcatgagattactggcagcaaaggcgacttcatagtggctgaccacacccagatgaacactcccattggtggaggtccagttcatgttccagagtatcatcacatgtcttaccatgtgaaactttccaaagatgtgacagaccacagagacaacatgtccttgaaagaaactgtcagagctgttgactgtcgcaagacctacctt

SEQ ID NO: 21 - DNA, 218 bp, Diabrotica virgerifera
tagctctgatgacagagcccatcgagtttcaagccaaacagttgcataaagctatcagcggattgggaactgatgaaagtacaatmgtmgaaattttaagtgtmcacaacaacgatgagattataagaatttcccaggcctatgaaggattgtaccaacgmtcattggaatctgatatcaaaggagatacctcaggaacattaaaaaagaattattag

SEQ ID NO: 22 - DNA, 424 bp, Diabrotica virgerifera
  misc_feature (393)..(393): n is a, c, g, or t
  misc_feature (394)..(394): n is a, c, g, or t
  misc_feature (395)..(395): n is a, c, g, or t
ttgttacaagctggagaacttctctttgctggaaccgaagagtcagtatttaatgctgtattctgtcaaagaaataaaccacaattgaatttgatattcgacaaatatgaagaaattgttgggcatcccattgaaaaagccattgaaaacgagttttcaggaaatgctaaacaagccatgttacaccttatccagagcgtaagagatcaagttgcatatttggtaaccaggctgcatgattcaatggcaggcgtcggtactgacgatagaactttaatcagaattgttgtttcgagatctgaaatcgatctagaggaaatcaaacaatgctatgaagaaatctacagtaaaaccttggctgataggatagcggatgacacatctggcgactannnaaaagccttattagccgttgttggttaag

SEQ ID NO: 23 - DNA, 397 bp, Diabrotica virgerifera
agatgttggctgcatctagagaattacacaagttcttccatgattgcaaggatgtactgagcagaatagtggaaaaacaggtatccatgtctgatgaattgggaagggacgcaggagctgtcaatgcccttcaacgcaaacaccagaacttcctccaagacctacaaacactccaatcgaacgtccaacaaatccaagaagaatcagctaaacttcaagctagctatgccggtgatagagctaaagaaatcaccaacagggagcaggaagtggtagcagcctgggcagccttgcagatcgcttgcgatcagagacacggaaaattgagcgatactggtgatctattcaaattctttaacttggtacgaacgttgatgcagtggatggacgaatggac

SEQ ID NO: 24 - DNA, 490 bp, Diabrotica virgerifera
gcagatgaacaccagcgagaaaccaagagatgttagtggtgttgaattgttgatgaacaaccatcagacactcaaggctgagatcgaagccagagaagacaactttacggcttgtatttctttaggaaaggaattgttgagccgtaatcactatgctagtgctgatattaaggataaattggtcgcgttgacgaatcaaaggaatgctgtactacagaggtgggaagaaagatgggagaacttgcaactcatcctcgaggtataccaattcgccagagatgcggccgtcgccgaagcatggttgatcgcacaagaaccttacttgatgagccaagaactaggacacaccattgacgacgttgaaaacttgataaagaaacacgaagcgttcgaaaaatcggcagcggcgcaagaagagagattcagtgctttggagagactgacgacgttcgaattgagagaaataaagaggaaacaagaagctgcccag

SEQ ID NO: 25 - DNA, 330 bp, Diabrotica virgerifera
agtgaaatgttagcaaatataacatccaagtttcgtaattgtacttgctcagttagaaaatattctgtagtttcactatcttcaaccgaaaatagaataaatgtagaacctcgcgaacttgcctttcctccaaaatatcaagaacctcgacaagtttggttggagagtttagatacgatagacgacaaaaaattgggtattcttgagctgcatcctgatgtttttgctactaatccaagaatagatattatacatcaaaatgttagatggcaaagtttatatagatatgtaagctatgctcatacaaagtcaagatttgaagtgagaggt

SEQ ID NO: 26 - DNA, 320 bp, Diabrotica virgerifera
caaagtcaagatttgaagtgagaggtggaggtcgaaaaccgtggccgcaaaagggattgggacgtgctcgacatggttcaattagaagtccactttggagaggtggaggagttgttcatggaccaaaatctccaacccctcatttttacatgattccattctacacccgtttgctgggtttgactagcgcactttcagtaaaatttgcccaagatgacttgcacgttgtggatagtctagatctgccaactgacgaacaaagttatatagaagagctggtcaaaagccgcttttgggggtccttcttgttttatttgtag

SEQ ID NO: 27 - DNA, 46 bp, Artificial Sequence
  Ann-F1_T7 PCR Primer Oligonucleotide
ttaatacgactcactatagggagagctccaacagtggttccttatc

SEQ ID NO: 28 - DNA, 29 bp, Artificial Sequence
  Ann-R1 PCR Primer Oligonucleotide
ctaataattcttttttaatgttcctgagg

SEQ ID NO: 29 - DNA, 22 bp, Artificial Sequence
  Ann-F1 PCR Primer Oligonucleotide
gctccaacagtggttccttatc

SEQ ID NO: 30 - DNA, 53 bp, Artificial Sequence
  Ann-R1_T7 PCR Primer Oligonucleotide
ttaatacgactcactatagggagactaataattcttttttaatgttcctgagg

SEQ ID NO: 31 - DNA, 48 bp, Artificial Sequence
  Ann-F2_T7 PCR Primer Oligonucleotide
ttaatacgactcactatagggagattgttacaagctggagaacttctc

SEQ ID NO: 32 - DNA, 24 bp, Artificial Sequence
  Ann-R2 PCR Primer Oligonucleotide
cttaaccaacaacggctaataagg

SEQ ID NO: 33 - DNA, 24 bp, Artificial Sequence
  Ann-F2 PCR Primer Oligonucleotide
ttgttacaagctggagaacttctc

SEQ ID NO: 34 - DNA, 48 bp, Artificial Sequence
  Ann-R2T7 PCR Primer Oligonucleotide
ttaatacgactcactatagggagacttaaccaacaacggctaataagg

SEQ ID NO: 35 - DNA, 47 bp, Artificial Sequence
  Betasp2-F1_T7 PCR Primer Oligonucleotide
ttaatacgactcactatagggagaagatgttggctgcatctagagaa

SEQ ID NO: 36 - DNA, 22 bp, Artificial Sequence
  Betasp2-R1 PCR Primer Oligonucleotide
gtccattcgtccatccactgca

SEQ ID NO: 37 - DNA, 23 bp, Artificial Sequence
  Betasp2-F1 PCR Primer Oligonucleotide
agatgttggctgcatctagagaa

SEQ ID NO: 38 - DNA, 46 bp, Artificial Sequence
  Betasp2-R1_T7 PCR Primer Oligonucleotide
ttaatacgactcactatagggagagtccattcgtccatccactgca

SEQ ID NO: 39 - DNA, 46 bp, Artificial Sequence
  Betasp2-F2_T7 PCR Primer Oligonucleotide
ttaatacgactcactatagggagagcagatgaacaccagcgagaaa

SEQ ID NO: 40 - DNA, 22 bp, Artificial Sequence
  Betasp2-R2 PCR Primer Oligonucleotide
ctgggcagcttcttgtttcctc

SEQ ID NO: 41 - DNA, 22 bp, Artificial Sequence
  Betasp2-F2 PCR Primer Oligonucleotide
gcagatgaacaccagcgagaaa

SEQ ID NO: 42 - DNA, 46 bp, Artificial Sequence
  Betasp2-R2_T7 PCR Primer Oligonucleotide
ttaatacgactcactatagggagactgggcagcttcttgtttcctc

SEQ ID NO: 43 - DNA, 51 bp, Artificial Sequence
  L4-F1_T7 PCR Primer Oligonucleotide
ttaatacgactcactatagggagaagtgaaatgttagcaaatataacatcc

SEQ ID NO: 44 - DNA, 26 bp, Artificial Sequence
  L4-R1 PCR Primer Oligonucleotide
acctctcacttcaaatcttgactttg

SEQ ID NO: 45 - DNA, 27 bp, Artificial Sequence
  L4-F1 PCR Primer Oligonucleotide
agtgaaatgttagcaaatataacatcc

SEQ ID NO: 46 - DNA, 50 bp, Artificial Sequence
  L4-R1_T7 PCR Primer Oligonucleotide
ttaatacgactcactatagggagaacctctcacttcaaatcttgactttg

SEQ ID NO: 47 - DNA, 50 bp, Artificial Sequence
  L4-F2_T7 PCR Primer Oligonucleotide
ttaatacgactcactatagggagacaaagtcaagatttgaagtgagaggt

SEQ ID NO: 48 - DNA, 25 bp, Artificial Sequence
  L4-R2 PCR Primer Oligonucleotide
ctacaaataaaacaagaaggacccc

SEQ ID NO: 49 - DNA, 26 bp, Artificial Sequence
  L4-F2 PCR Primer Oligonucleotide
caaagtcaagatttgaagtgagaggt

SEQ ID NO: 50 - DNA, 49 bp, Artificial Sequence
  L4-R2_T7 PCR Primer Oligonucleotide
ttaatacgactcactatagggagactacaaataaaacaagaaggacccc

SEQ ID NO: 51 - DNA, 1150 bp, Zea mays
caacggggcagcactgcactgcactgcaactgcgaatttccgtcagcttggagcggtccaagcgccctgcgaagcaaactacgccgatggcttcggcggcggcgtgggagggtccgacggccgcggagctgaagacagcgggggcggaggtgattcccggcggcgtgcgagtgaaggggtgggtcatccagtcccacaaaggccctatcctcaacgccgcctctctgcaacgctttgaagatgaacttcaaacaacacatttacctgagatggtttttggagagagtttcttgtcacttcaacatacacaaactggcatcaaatttcattttaatgcgcttgatgcactcaaggcatggaagaaagaggcactgccacctgttgaggttcctgctgcagcaaaatggaagttcagaagtaagccttctgaccaggttatacttgactacgactatacatttacgacaccatattgtgggagtgatgctgtggttgtgaactctggcactccacaaacaagtttagatggatgcggcactttgtgttgggaggatactaatgatcggattgacattgttgccctttcagcaaaagaacccattcttttctacgacgaggttatcttgtatgaagatgagttagctgacaatggtatctcatttcttactgtgcgagtgagggtaatgccaactggttggtttctgcttttgcgtttttggcttagagttgatggtgtactgatgaggttgagagacactcggttacattgcctgtttggaaacggcgacggagccaagccagtggtacttcgtgagtgctgctggagggaagcaacatttgctactttgtctgcgaaaggatatccttcggactctgcagcgtacgcggacccgaaccttattgcccataagcttcctattgtgacgcagaagacccaaaagctgaaaaatcctacctgactgacacaaaggcgccctaccgcgtgtacatcatgactgtcctgtcctatcgttgccttttgtgtttgccacatgttgtggatgtacgtttctatgacgaaacaccatagtccatttcgcctgggccgaacagagatagctgattgtcatgtcacgtttgaattagaccattccttagccctttttccccc

SEQ ID NO: 52 - DNA, 22 bp, Artificial Sequence
  T20NV PCR Primer Oligonucleotide
  misc_feature (22)..(22): n is a, c, g, or t
ttttttttttttttttttttvn

SEQ ID NO: 53 - DNA, 20 bp, Artificial Sequence
  P5U76S (F) PCR Primer Oligonucleotide
ttgtgatgttggtggcgtat

SEQ ID NO: 54 - DNA, 24 bp, Artificial Sequence
  P5U76A (R) PCR Primer Oligonucleotide
tgttaaataaaaccccaaagatcg

SEQ ID NO: 55 - DNA, 21 bp, Artificial Sequence
  TIPmxF PCR Primer Oligonucleotide
tgagggtaatgccaactggtt

SEQ ID NO: 56 - DNA, 24 bp, Artificial Sequence
  TIPmxR PCR Primer Oligonucleotide
gcaatgtaaccgagtgtctctcaa

SEQ ID NO: 57 - DNA, 32 bp, Artificial Sequence
  HXTIP Probe Oligonucleotide
tttttggcttagagttgatggtgtactgatga

SEQ ID NO: 58 - DNA, 151 bp, Artificial Sequence
  Portion of SpecR coding region
gaccgtaaggcttgatgaaacaacgcggcgagctttgatcaacgaccttttggaaacttcggcttcccctggagagagcgagattctccgcgctgtagaagtcaccattgttgtgcacgacgacatcattccgtggcgttatccagctaag

SEQ ID NO: 59 - DNA, 69 bp, Artificial Sequence
  Portion of AAD1 coding region
tgttcggttccctctaccaagcacagaaccgtcgcttcagcaacacctcagtcaaggtgatggatgttg

SEQ ID NO: 60 - DNA, 4233 bp, Zea mays
agcctggtgtttccggaggagacagacatgatccctgccgttgctgatccgacgacgctggacggcgggggcgcgcgcaggccgttgctcccggagacggaccctcgggggcgtgctgccgccggcgccgagcagaagcggccgccggctacgccgaccgttctcaccgccgtcgtctccgccgtgctcctgctcgtcctcgtggcggtcacagtcctcgcgtcgcagcacgtcgacgggcaggctgggggcgttcccgcgggcgaagatgccgtcgtcgtcgaggtggccgcctcccgtggcgtggctgagggcgtgtcggagaagtccacggccccgctcctcggctccggcgcgctccaggacttctcctggaccaacgcgatgctggcgtggcagcgcacggcgttccacttccagccccccaagaactggatgaacggttagttggacccgtcgccatcggtgacgacgcgcggatcgtttttttcttttttcctctcgttctggctctaacttggttccgcgtttctgtcacggacgcctcgtgcacatggcgatacccgatccgccggccgcgtatatctatctacctcgaccggcttctccagatccgaacggtaagttgttggctccgatacgatcgatcacatgtgagctcggcatgctgcttttctgcgcgtgcatgcggctcctagcattccacgtccacgggtcgtgacatcaatgcacgatataatcgtatcggtacagagatattgtcccatcagctgctagctttcgcgtattgatgtcgtgacattttgcacgcaggtccgctgtatcacaagggctggtaccacctcttctaccagtggaacccggactccgcggtatggggcaacatcacctggggccacgccgtctcgcgcgacctcctccactggctgcacctaccgctggccatggtgcccgatcacccgtacgacgccaacggcgtctggtccgggtcggcgacgcgcctgcccgacggccggatcgtcatgctctacacgggctccacggcggagtcgtcggcgcaggtgcagaacctcgcggagccggccgacgcgtccgacccgctgctgcgggagtgggtcaagtcggacgccaacccggtgctggtgccgccgccgggcatcgggccgacggacttccgcgacccgacgacggcgtgtcggacgccggccggcaacgacacggcgtggcgggtcgccatcgggtccaaggaccgggaccacgcggggctggcgctggtgtaccggacggaggacttcgtgcggtacgacccggcgccggcgctgatgcacgccgtgccgggcaccggcatgtgggagtgcgtggacttctacccggtggccgcgggatcaggcgccgcggcgggcagcggggacgggctggagacgtccgcggcgccgggacccggggtgaagcacgtgctcaaggctagcctcgacgacgacaagcacgactactacgcgatcggcacctacgacccggcgacggacacctggacccccgacagcgcggaggacgacgtcgggatcggcctccggtacgactatggcaagtactacgcgtcgaagaccttctacgaccccgtccttcgccggcgggtgctctgggggtgggtcggcgagaccgacagcgagcgcgcggacatcctcaagggctgggcatccgtgcaggtacgtctcagggtttgaggctagcatggcttcaatcttgctggcatcgaatcattaatgggcagatattataacttgataatctgggttggttgtgtgtggtggggatggtgacacacgcgcggtaataatgtagctaagctggttaaggatgagtaatggggttgcgtataaacgacagctctgctaccattacttctgacacccgattgaaggagacaacagtaggggtagccggtagggttcgtcgacttgccttttcttttttcctttgttttgttgtggatcgtccaacacaaggaaaataggatcatccaacaaacatggaagtaatcccgtaaaacatttctcaaggaaccatctagctagacgagcgtggcatgatccatgcatgcacaaacactagataggtctctgcagctgtgatgttcctttacatataccaccgtccaaactgaatccggtctgaaaattgttcaagcagagaggccccgatcctcacacctgtacacgtccctgtacgcgccgtcgtggtctcccgtgatcctgccccgtcccctccacgcggccacgcctgctgcagcgctctgtacaagcgtgcaccacgtgagaatttccgtctactcgagcctagtagttagacgggaaaacgagaggaagcgcacggtccaagcacaacactttgcgcgggcccgtgacttgtctccggttggctgagggcgcgcgacagagatgtatggcgccgcggcgtgtcttgtgtcttgtcttgcctatacaccgtagtcagagactgtgtcaaagccgtccaacgacaatgagctaggaaacgggttggagagctgggttcttgccttgcctcctgtgatgtctttgccttgcatagggggcgcagtatgtagctttgcgttttacttcacgccaaaggatactgctgatcgtgaattattattattatatatatatcgaatatcgatttcgtcgctctcgtggggttttattttccagactcaaacttttcaaaaggcctgtgttttagttcttttcttccaattgagtaggcaaggcgtgtgagtgtgaccaacgcatgcatggatatcgtggtagactggtagagctgtcgttaccagcgcgatgcttgtatatgtttgcagtattttcaaatgaatgtctcagctagcgtacagttgaccaagtcgacgtggagggcgcacaacagacctctgacattattcactttttttttaccatgccgtgcacgtgcagtcaatccccaggacggtcctcctggacacgaagacgggcagcaacctgctccagtggccggtggtggaggtggagaacctccggatgagcggcaagagcttcgacggcgtcgcgctggaccgcggatccgtcgtgcccctcgacgtcggcaaggcgacgcaggtgacgccgcacgcagcctgctgcagcgaacgaactcgcgcgttgccggcccgcggccagctgacttagtttctctggctgatcgaccgtgtgcctgcgtgcgtgcagttggacatcgaggctgtgttcgaggtggacgcgtcggacgcggcgggcgtcacggaggccgacgtgacgttcaactgcagcaccagcgcaggcgcggcgggccggggcctgctcggcccgttcggccttctcgtgctggcggacgacgacttgtccgagcagaccgccgtgtacttctacctgctcaagggcacggacggcagcctccaaactttcttctgccaagacgagctcaggtatgtatgttatgacttatgaccatgcatgcatgcgcatttcttagctaggctgtgaagcttcttgttgagttgtttcacagatgcttaccgtctgctttgtttcgtatttcgactaggcatccaaggcgaacgatctggttaagagagtatacgggagcttggtccctgtgctagatggggagaatctctcggtcagaatactggtaagtttttacagcgccagccatgcatgtgttggccagccagctgctggtactttggacactcgttcttctcgcactgctcattattgcttctgatctggatgcactacaaattgaaggttgaccactccatcgtggagagctttgctcaaggcgggaggacgtgcatcacgtcgcgagtgtaccccacacgagccatctacgactccgcccgcgtcttcctcttcaacaacgccacacatgctcacgtcaaagcaaaatccgtcaagatctggcagctcaactccgcctacatccggccatatccggcaacgacgacttctctatgactaaattaagtgacggacagataggcgatattgcatacttgcatcatgaactcatttgtacaacagtgattgtttaatttatttgctgccttccttatccttcttgtgaaactatatggtacacacatgtatcattaggtctagtagtgttgttgcaaagacacttagacaccagaggttccaggagtatcagagataaggtataagagggagcagggagcag

SEQ ID NO: 61 - DNA, 25 bp, Artificial Sequence
  ST-LS1- F PCR Primer Oligonucleotide
gtatgtttctgcttctacctttgat

SEQ ID NO: 62 - DNA, 29 bp, Artificial Sequence
  ST-LS1- R PCR Primer Oligonucleotide
ccatgttttggtcatatattagaaaagtt

SEQ ID NO: 63 - DNA, 34 bp, Artificial Sequence
  ST-LS1-P Probe Oligonucleotide
agtaatatagtatttcaagtatttttttcaaaat

SEQ ID NO: 64 - DNA, 20 bp, Artificial Sequence
  GAAD1-F PCR Primer Oligonucleotide
tgttcggttccctctaccaa

SEQ ID NO: 65 - DNA, 22 bp, Artificial Sequence
  GAAD1-R PCR Primer Oligonucleotide
caacatccatcaccttgactga

SEQ ID NO: 66 - DNA, 24 bp, Artificial Sequence
  GAAD1-P Probe Oligonucleotide
cacagaaccgtcgcttcagcaaca

SEQ ID NO: 67 - DNA, 18 bp, Artificial Sequence
  IVR1-F PCR Primer Oligonucleotide
tggcggacgacgacttgt

SEQ ID NO: 68 - DNA, 19 bp, Artificial Sequence
  IVR1-R PCR Primer Oligonucleotide
aaagtttggaggctgccgt

SEQ ID NO: 69 - DNA, 26 bp, Artificial Sequence
  IVR1-P Probe Oligonucleotide
cgagcagaccgccgtgtacttctacc

SEQ ID NO: 70 - DNA, 19 bp, Artificial Sequence
  SPC1A PCR Primer Oligonucleotide
cttagctggataacgccac

SEQ ID NO: 71 - DNA, 19 bp, Artificial Sequence
  SPC1S PCR Primer Oligonucleotide
gaccgtaaggcttgatgaa

SEQ ID NO: 72 - DNA, 21 bp, Artificial Sequence
  TQSPEC Probe Oligonucleotide
cgagattctccgcgctgtaga

SEQ ID NO: 73 - DNA, 3093 bp, Meligethes aeneus
gagacccaacaccagaagactttcatagggaaaatcccgattatgttgaggtctacgtactgccttctcagcggcttaacagatcgtgatttgacggagttaaacgagtgtcctttggatcccgggggttatttcatcataaacgggtcggagaaggttttaattgcccaggaaaaaatggctacgaacacagtgtatgtgttttcgatgaaggacgggaaatacgcgtttaaatccgagattaggtcgtgtttggagcattcttcgcgccccacctccactttgtgggtgaatatgatggctcgtggcgggcaagctgtgaaaaaggcagccatcgggcaaagaatcatcgctattttaccatatatcaagcaagaaatacccattatgatcgtattcagagcgctaggttttgtggccgacagagacatcctcgaacacatcatctatgactttgacgaccctgaaatgatggagatggtgaaaccgtccctagacgaggcttttgtaatccaagagcagggtgtggccttgaattttattggtgctagaggggccaggcccggcgtaacgagggaaaagcgtgttaaatacgccagggaaattttgcagaaggaaatgctgccgcatgtaggagtttccgatttctgcgaaaccaaaaaagcgtatttcttggggtacatggtgcacaggctgcttctggcctctttggggcgcagagagttagacgacagggatcattacggcaacaaaaggttggatttggctgggccgttgctggctttcttgttcagaggtcttttcaaaaacttaatgaaggaagtgcgcatgtacgcccaaaaattcatcgacagaggaaaagatttcaacttggatttggcaatcaaaaccaaactcatcaccgacggtttgcgttactctcttgccaccggtaactggggcgaccagaaaaaggcccatcaagccagagccggagtgtctcaggtactgaacagactgacttacgcctcgactttatctcatttgaggcgcgtaaactcgcccatcggtcgcgacggtaaactagccaaaccccgtcagttgcacaacaccctgtggggcatgatttgcccggcggaaacgccagagggcgctgcggtgggtttggtaaaaaatctcgcccttatggcttacatttccgtcggttcgcaaccctctccgatcttggagttcttggaggagtggtcgatggagaatttggaggaaatagcgccgtctgctatcgctaacgccactaagatttttgtcaatgggtgttgggtcggtattcacagggatccggagcaattgacggcgactttgaggaagctacgtcgccagatggatattatcgtatccgaggtatccatgatccgtgatatccgcgatcgcgaaatccgtatctacacggatgctggtcgtatttgcagacctttattgattgctaaaaatggcagcctgttactgaaaaaagaacacatcgacatgttgaaagagagagaatacaacaactatggctggcaagtgttggtagcctcaggtgttgtcgaatacattgacaccctagaagaagaaactgtgatgattgccatgtctcctgacgatttgagacaagacaaggagtgcgcctactgtacgacttacactcactgcgaaattcatcccgccatgattttgggagtctgcgcgtcaattatcccgttccccgatcacaaccaaagtcccaggaacacctatcaaagcgccatgggaaaacaagccatgggcgtgtacataacaaacttccacgtgcggatggacacgctcgcgcacgtgctctactacccccacaaaccgctggtaaccaccagatccatggagtacctgcggttcagagagcttcccgccggcatcaacagcatcgtggccatcgcctgctacaccggctacaaccaggaggattcggttattttaaacgcttcggccgtcgaaagaggcttcttccgatcggtgttttatcgttcgtacaaggacgccgagtccaagcgcattggggatcaggaggagcagttcgagaagccgaccaggcagacctgccagggcatgcgcaacgcgctgtacgacaaactcgacgacgacggtatcatttcgcccggtattcgtgtctccggggacgacgtcgtcatcggcaaaaccatgacactcccggaaaacgacgatgagctggacggtaacacgaagaagttcaccaagagggacgccagtactttcttgcgtaacagcgagactggcgtggtggatcaggtgatgttgaccttgaactccgagggttacaagttctgtaagattcgcgtgaggtccgtgaggattccgcagataggcgacaaattcgcctcgcgtcacgggcagaagggtacttgcggcatacagtaccggcaagaagatatgattttctcgtgcgagggtttgaccccggacatcatcatcaacccgcacgccatcccatctcgtatgacgattgggcatttgatcgagtgcatccaaggtaaggtatcggcgaataagggggagatcggggacgcgaccccgtttaacgacgcggtaaacgtgcagaaaatttccactctcctgcaagagtacgggtaccaactgagagggaacgaggtgatgtacaacgggcacacggggcgcaaaatgaacgcgcagattttcctgggccccacctactaccagcgcctcaagcacatggtggacgataagatccactcgagggccagaggcccggtgcagatcctcgtcaggcagcccatggagggtcgagccagggacgggggcctgcgtttcggggagatggagcgcgattgccagatttcgcacggcgcggcgcagtttctgcgcgagcgcttgttcgaggtgtccgatccctacaggatccacgtgtgcaacttctgcgggctgatcgccatcgctaacttgcggaacaacacgttcgagtgcaaggggtgcaagaataagacgcagatttcgcagacatggatcctgtagggatcggacacctcgaacaagcgctcgcgcagaaactgcgccgcgccgtgc

SEQ ID NO: 74 - protein, 1013 aa, Meligethes aeneus
ETQHQKTFIGKIPIMLRSTYCLLSGLTDRDLTELNECPLDPGGYFIINGSEKVLIAQEKMATNTVYVFSMKDGKYAFKSEIRSCLEHSSRPTSTLWVNMMARGGQAVKKAAIGQRIIAILPYIKQEIPIMIVFRALGFVADRDILEHIIYDFDDPEMMEMVKPSLDEAFVIQEQGVALNFIGARGARPGVTREKRVKYAREILQKEMLPHVGVSDFCETKKAYFLGYMVHRLLLASLGRRELDDRDHYGNKRLDLAGPLLAFLFRGLFKNLMKEVRMYAQKFIDRGKDFNLDLAIKTKLITDGLRYSLATGNWGDQKKAHQARAGVSQVLNRLTYASTLSHLRRVNSPIGRDGKLAKPRQLHNTLWGMICPAETPEGAAVGLVKNLALMAYISVGSQPSPILEFLEEWSMENLEEIAPSAIANATKIFVNGCWVGIHRDPEQLTATLRKLRRQMDIIVSEVSMIRDIRDREIRIYTDAGRICRPLLIAKNGSLLLKKEHIDMLKEREYNNYGWQVLVASGVVEYIDTLEEETVMIAMSPDDLRQDKECAYCTTYTHCEIHPAMILGVCASIIPFPDHNQSPRNTYQSAMGKQAMGVYITNFHVRMDTLAHVLYYPHKPLVTTRSMEYLRFRELPAGINSIVAIACYTGYNQEDSVILNASAVERGFFRSVFYRSYKDAESKRIGDQEEQFEKPTRQTCQGMRNALYDKLDDDGIISPGIRVSGDDVVIGKTMTLPENDDELDGNTKKFTKRDASTFLRNSETGVVDQVMLTLNSEGYKFCKIRVRSVRIPQIGDKFASRHGQKGTCGIQYRQEDMIFSCEGLTPDIIINPHAIPSRMTIGHLIECIQGKVSANKGEIGDATPFNDAVNVQKISTLLQEYGYQLRGNEVMYNGHTGRKMNAQIFLGPTYYQRLKHMVDDKIHSRARGPVQILVRQPMEGRARDGGLRFGEMERDCQISHGAAQFLRERLFEVSDPYRIHVCNFCGLIAIANLRNNTFECKGCKNKTQISQTWIL

SEQ ID NO: 75 - DNA, 2279 bp, Meligethes aeneus
gagacccaacaccagaagactttcatagggaaaatcccgattatgttgaggtctacgtactgccttctcagcggcttaacagatcgtgatttgacggagttaaacgagtgtcctttggatcccgggggttatttcatcataaacgggtcggagaaggttttaattgcccaggaaaaaatggctacgaacacagtgtatgtgttttcgatgaaggacgggaaatacgcgtttaaatccgagattaggtcgtgtttggagcattcttcgcgccccacctccactttgtgggtgaacatgatggcccgtggtgggcaggctgtcaaaaaggcggccatcgggcaaagaattattgccattttaccatatatcaagcaagaaatacccattatgatcgtattcagagcgttgggttttgtggctgacagagatatcctggaacacatcatttatgactttgacgaccctgaaatgatggagatggtgaaaccgtccctggacgaggcctttgtaattcaagagcagggtgtggctttgaattttatcggggctagaggggccaggcccggcgtaacgagggaaaagcgtgttaaatacgccagggaaattttgcagaaggaaatgctgccgcatgtaggagtttccgatttctgcgaaaccaaaaaagcgtatttcttggggtacatggtgcacaggctgcttctggcctctttggggcgcagagagttagacgacagggatcattacggcaacaaaaggttggatttggctgggccgttgctggctttcttgttcagaggtcttttcaaaaacttaatgaaggaagtgcgcatgtacgcccaaaaattcatcgacagaggaaaagatttcaacttggatttggcaatcaaaaccaaactcatcaccgacggtttgcgttactctcttgccaccggtaactggggcgaccagaaaaaggcccatcaagccagagccggagtgtctcaggtactgaacagactgacttacgcctcgactttatctcatttgaggcgcgtaaactcgcccatcggtcgcgacggtaaactagccaaaccccgtcagttgcacaacaccctgtggggcatgatttgcccggcggaaacgccagagggcgctgcggtgggtttggtaaaaaatctcgcccttatggcttacatttccgtcggttcgcaaccctctccgatcttggagttcttggaggagtggtcgatggagaatttggaggaaatagcgccgtctgctatcgctaacgccactaagatttttgtcaatgggtgttgggtcggtattcacagggatccggagcaattgacggcgactttgaggaagctacgtcgccagatggatattatcgtatccgaggtatccatgatccgtgatatccgcgatcgcgaaatccgtatctacacggatgctggtcgtatttgcagacctttattgattgctaaaaatggcagcctgttactgaaaaaagaacacatcgacatgttgaaagagagagaatacaacaactatggctggcaagtgttggtagcctcaggtgttgtcgaatacattgacaccctagaagaagaaactgtgatgattgccatgtctcctgacgatttgagacaagacaaggagtgcgcctactgtacgacttacactcactgcgaaattcatcccgccatgattttgggagtctgcgcgtcaattatcccgttccccgatcacaaccaaagtcccaggaacacctatcaaagcgccatgggaaaacaagccatgggcgtgtacataacaaacttccacgtgcggatggacacgctcgcgcacgtgctctactacccccacaaaccgctggtaaccaccagatccatggagtacctgcggttcagagagctccccgccggcatcaacagcatcgtggccatcgcctgctacaccggctacaaccaggaagattcggttatattgaacgcttcggccgtcgaaagaggcttcttccggtcggtgttctaccgttcgtacaaggacgccgagtccaaacggatcggggatcaggaggagcagttcgagaagccgaccaggcagacctgccagggcatgcgcaacgcgctgtacgacaaattggacgacgacggcataatttcgcctggcatccgtgtttccggggacgatgtcgtcataggcaaaaccatgacactcccggagaacgatgatgagctggacggtaacacgaagaagttcaccaagagggacgccagtactttcttgcgtaacag

SEQ ID NO: 76 - protein, 759 aa, Meligethes aeneus
ETQHQKTFIGKIPIMLRSTYCLLSGLTDRDLTELNECPLDPGGYFIINGSEKVLIAQEKMATNTVYVFSMKDGKYAFKSEIRSCLEHSSRPTSTLWVNMMARGGQAVKKAAIGQRIIAILPYIKQEIPIMIVFRALGFVADRDILEHIIYDFDDPEMMEMVKPSLDEAFVIQEQGVALNFIGARGARPGVTREKRVKYAREILQKEMLPHVGVSDFCETKKAYFLGYMVHRLLLASLGRRELDDRDHYGNKRLDLAGPLLAFLFRGLFKNLMKEVRMYAQKFIDRGKDFNLDLAIKTKLITDGLRYSLATGNWGDQKKAHQARAGVSQVLNRLTYASTLSHLRRVNSPIGRDGKLAKPRQLHNTLWGMICPAETPEGAAVGLVKNLALMAYISVGSQPSPILEFLEEWSMENLEEIAPSAIANATKIFVNGCWVGIHRDPEQLTATLRKLRRQMDIIVSEVSMIRDIRDREIRIYTDAGRICRPLLIAKNGSLLLKKEHIDMLKEREYNNYGWQVLVASGVVEYIDTLEEETVMIAMSPDDLRQDKECAYCTTYTHCEIHPAMILGVCASIIPFPDHNQSPRNTYQSAMGKQAMGVYITNFHVRMDTLAHVLYYPHKPLVTTRSMEYLRFRELPAGINSIVAIACYTGYNQEDSVILNASAVERGFFRSVFYRSYKDAESKRIGDQEEQFEKPTRQTCQGMRNALYDKLDDDGIISPGIRVSGDDVVIGKTMTLPENDDELDGNTKKFTKRDASTFLRN

SEQ ID NO: 77 - DNA, 447 bp, Meligethes aeneus
ccgacggtttgcgttactctcttgccaccggtaactggggcgaccagaaaaaggcccatcaagccagagccggagtgtctcaggtattgaacagactgacttacgcctcgactttatctcatttgaggcgcgtaaactcgcccatcggtcgcgacggtaaattagccaaaccccgtcagttgcacaacaccctgtggggcatgatttgcccggcggaaacgccagagggcgctgcggtgggtttggtaaaaaatctcgcccttatggcttacatttccgtcggttcgcaaccctctccgatcttggagttcttggaggagtggtcgatggagaatttggaggaaatagcgccgtctgctatcgctaacgccactaagatttttgtcaatgggtgttgggtcggtattcacagggatccggagcaattgacggcgactttgaggaaac

SEQ ID NO: 78 - DNA, 44 bp, Artificial Sequence
  forward primer to amplify RpII140
taatacgactcactatagggagagtttcctcaaagtcgccgtca

SEQ ID NO: 79 - DNA, 44 bp, Artificial sequence
  reverse primer to amplify RpII140
taatacgactcactatagggagaccgacggtttgcgttactctc

SEQ ID NO: 80 - protein, 999 aa, Meligethes aeneus
MLRSTYCLLSGLTDRDLTELNECPLDPGGYFIINGSEKVLIAQEKMATNTVYVFSMKDGKYAFKSEIRSCLEHSSRPTSTLWVNMMARGGQAVKKAAIGQRIIAILPYIKQEIPIMIVFRALGFVADRDILEHIIYDFDDPEMMEMVKPSLDEAFVIQEQGVALNFIGARGARPGVTREKRVKYAREILQKEMLPHVGVSDFCETKKAYFLGYMVHRLLLASLGRRELDDRDHYGNKRLDLAGPLLAFLFRGLFKNLMKEVRMYAQKFIDRGKDFNLDLAIKTKLITDGLRYSLATGNWGDQKKAHQARAGVSQVLNRLTYASTLSHLRRVNSPIGRDGKLAKPRQLHNTLWGMICPAETPEGAAVGLVKNLALMAYISVGSQPSPILEFLEEWSMENLEEIAPSAIANATKIFVNGCWVGIHRDPEQLTATLRKLRRQMDIIVSEVSMIRDIRDREIRIYTDAGRICRPLLIAKNGSLLLKKEHIDMLKEREYNNYGWQVLVASGVVEYIDTLEEETVMIAMSPDDLRQDKECAYCTTYTHCEIHPAMILGVCASIIPFPDHNQSPRNTYQSAMGKQAMGVYITNFHVRMDTLAHVLYYPHKPLVTTRSMEYLRFRELPAGINSIVAIACYTGYNQEDSVILNASAVERGFFRSVFYRSYKDAESKRIGDQEEQFEKPTRQTCQGMRNALYDKLDDDGIISPGIRVSGDDVVIGKTMTLPENDDELDGNTKKFTKRDASTFLRNSETGVVDQVMLTLNSEGYKFCKIRVRSVRIPQIGDKFASRHGQKGTCGIQYRQEDMIFSCEGLTPDIIINPHAIPSRMTIGHLIECIQGKVSANKGEIGDATPFNDAVNVQKISTLLQEYGYQLRGNEVMYNGHTGRKMNAQIFLGPTYYQRLKHMVDDKIHSRARGPVQILVRQPMEGRARDGGLRFGEMERDCQISHGAAQFLRERLFEVSDPYRIHVCNFCGLIAIANLRNNTFECKGCKNKTQISQTWIL

SEQ ID NO: 81 - DNA, 3673 bp, Meligethes aeneus
cagattaaatcgcttttcggcggttgtgcttgtgtttttatttttgtgactttaaagatgtatgatcaagatgaagagcaatatgaggaggaagacgcggaagaaattagttccgaattgtggcaggaagcctgttggatcgttataaacgcgtatttcgacgagaaaggcctggtacggcaacaattggacagtttcgatgagttcattcagatgtctgtgcagagaatcgtggaggattccccgcaaatcgatttggtggcagaggcgcagcacacgtcgggagaagtggaaaaccccccgcgatatttgctgaaattcgagcagatttacctttcgaagcccacgcattgggagaaagacggggccccgtcccctatgatgcccaacgaggccagactgagaaatttgacgtactctgcacctctttacgtggacataacgaagactatcgttaaggagggcgaagatcctgtcgagacccaacaccagaagactttcatagggaaaatcccgattatgttgaggtctacgtactgccttctcagcggcttaacagatcgtgatttgacggagttaaacgagtgtcctttggatcccgggggttatttcatcataaacgggtcggagaaggttttaattgcccaggaaaaaatggctacgaacacagtgtatgtgttttcgatgaaggacgggaaatacgcgtttaaatccgagattaggtcgtgtttggagcattcttcgcgccccacctccactttgtgggtgaatatgatggctcgtggcgggcaagctgtgaaaaaggcagccatcgggcaaagaatcatcgctattttaccatatatcaagcaagaaatacccattatgatcgtattcagagcgctaggttttgtggccgacagagacatcctcgaacacatcatctatgactttgacgaccctgaaatgatggagatggtgaaaccgtccctagacgaggcttttgtaatccaagagcagggtgtggccttgaattttattggtgctagaggggccaggcccggcgtaacgagggaaaagcgtgttaaatacgccagggaaattttgcagaaggaaatgctgccgcatgtaggagtttccgatttctgtgaaaccaaaaaagcgtatttcttggggtacatggtgcacaggctgcttctggcctctttggggcgcagagagttagacgacagggatcattacggcaacaaaaggttggatttggctgggccgttgctggctttcttgttcagaggtcttttcaaaaacctaatgaaggaagtgcgaatgtacgcccaaaaattcatcgacagaggaaaagatttcaacttggatttggcaatcaaaaccaaactcatcaccgacggtttgcgttactctcttgccaccggtaactggggcgaccagaaaaaggcccatcaagccagagccggagtgtctcaggtattgaacagactgacttacgcctcgactttatctcatttgaggcgcgtaaactcgcccatcggtcgcgacggtaaattagccaaaccccgtcagttgcacaacaccctgtggggcatgatttgcccggcggaaacgccagagggcgctgcggtgggtttggtaaaaaatctcgcccttatggcttacatttccgtcggttcgcaaccttctccgatcttggagttcttggaggagtggtcgatggagaatttggaggaaatagcgccgtctgctatcgctaacgccactaagatttttgtcaatgggtgttgggtcggtattcacagggatccggagcaattgacggcgactttgaggaaactacgtcgccagatggatattatcgtatccgaggtatccatgatccgtgatatccgcgatcgcgaaatccgtatctacacggatgctggtcgcatttgcagacctttattgatcgccaaaaatggcagcctgttacttaaaaaagaacacatcgacatgttaaaagagagagaatacaacaactatggctggcaagtgttggtagcctcaggtgttgtcgaatacattgacaccctagaggaagaaactgtgatgattgccatgtctcctgacgatttgagacaagacaaggagtgcgcctactgtacgacttacactcactgcgaaattcatcccgccatgattttgggagtctgcgcgtcaattatcccgttccccgatcacaaccaaagtcccaggaacacctatcaaagcgccatgggaaaacaagccatgggcgtgtacataacaaacttccacgtgcggatggacacgctcgcgcacgtgctctactaccctcacaaaccgctggtaaccaccagatccatggagtacctccggttcagagagctccccgccggcatcaacagcatcgtggccatcgcctgctacaccggctacaaccaggaggattcggttattttaaacgcttcggccgtcgaaagaggcttcttccgatcggtgttttatcgttcgtacaaggacgccgagtccaagcgcattggggatcaggaggagcagttcgagaagccgaccaggcagacctgccagggcatgcggaacgcgctgtacgacaaactcgacgacgacggtatcatttcgcccggtattcgtgtctccggtgacgacgtcgtcatcggcaaaaccatgacgctcccggagaacgatgatgagctggacggtaacacgaagaagttcaccaagagggacgccagtactttcttgcgtaacagcgagactggcgtggtggatcaggtgatgttgacgttgaactccgagggttacaagttctgcaagatccgcgtgaggtccgtgaggattccgcagatcggcgacaagttcgcctcgcgtcacgggcagaagggtacttgcggcatacagtaccggcaagaagatatgattttctcgtgcgagggtttgaccccggacatcatcatcaacccgcacgccatcccatctcgtatgacgattgggcatttgatcgagtgcatccaaggtaaggtatcggcgaataagggggagatcggggacgcgaccccgtttaacgacgcggtaaacgtgcagaaaatttccactctcctgcaagagtacgggtaccaactgagagggaacgaggtgatgtacaacgggcacacggggcgcaaaatgaacgcgcagattttcctgggccccacctactaccagcgcctcaagcacatggtggacgacaagatccactcgagggccagaggcccggtgcagatcctcgtcaggcagcccatggagggtcgagccagggacgggggcctgcgtttcggggagatggagcgcgattgccagatttcgcacggcgcggcgcagtttctgcgcgagcgcttgttcgaggtgtccgatccctacaggatccacgtgtgcaacttctgcgggctgatcgccatcgccaacttgcggaacaacacgttcgagtgcaaggggtgcaagaataagacgcagatttcgcaggtcaagttgccttacgccgctaagttgctcttccaagagctgatgtcgatgaatatcgcccccagattgatggtcttataaaaagtttattttatgtattaggtattagaatttagttttgtattgattttatgtgactatgataccactaaaataaatataaatacaa

SEQ ID NO: 82 - protein, 1194 aa, Meligethes aeneus
QIKSLFGGCACVFIFVTLKMYDQDEEQYEEEDAEEISSELWQEACWIVINAYFDEKGLVRQQLDSFDEFIQMSVQRIVEDSPQIDLVAEAQHTSGEVENPPRYLLKFEQIYLSKPTHWEKDGAPSPMMPNEARLRNLTYSAPLYVDITKTIVKEGEDPVETQHQKTFIGKIPIMLRSTYCLLSGLTDRDLTELNECPLDPGGYFIINGSEKVLIAQEKMATNTVYVFSMKDGKYAFKSEIRSCLEHSSRPTSTLWVNMMARGGQAVKKAAIGQRIIAILPYIKQEIPIMIVFRALGFVADRDILEHIIYDFDDPEMMEMVKPSLDEAFVIQEQGVALNFIGARGARPGVTREKRVKYAREILQKEMLPHVGVSDFCETKKAYFLGYMVHRLLLASLGRRELDDRDHYGNKRLDLAGPLLAFLFRGLFKNLMKEVRMYAQKFIDRGKDFNLDLAIKTKLITDGLRYSLATGNWGDQKKAHQARAGVSQVLNRLTYASTLSHLRRVNSPIGRDGKLAKPRQLHNTLWGMICPAETPEGAAVGLVKNLALMAYISVGSQPSPILEFLEEWSMENLEEIAPSAIANATKIFVNGCWVGIHRDPEQLTATLRKLRRQMDIIVSEVSMIRDIRDREIRIYTDAGRICRPLLIAKNGSLLLKKEHIDMLKEREYNNYGWQVLVASGVVEYIDTLEEETVMIAMSPDDLRQDKECAYCTTYTHCEIHPAMILGVCASIIPFPDHNQSPRNTYQSAMGKQAMGVYITNFHVRMDTLAHVLYYPHKPLVTTRSMEYLRFRELPAGINSIVAIACYTGYNQEDSVILNASAVERGFFRSVFYRSYKDAESKRIGDQEEQFEKPTRQTCQGMRNALYDKLDDDGIISPGIRVSGDDVVIGKTMTLPENDDELDGNTKKFTKRDASTFLRNSETGVVDQVMLTLNSEGYKFCKIRVRSVRIPQIGDKFASRHGQKGTCGIQYRQEDMIFSCEGLTPDIIINPHAIPSRMTIGHLIECIQGKVSANKGEIGDATPFNDAVNVQKISTLLQEYGYQLRGNEVMYNGHTGRKMNAQIFLGPTYYQRLKHMVDDKIHSRARGPVQILVRQPMEGRARDGGLRFGEMERDCQISHGAAQFLRERLFEVSDPYRIHVCNFCGLIAIANLRNNTFECKGCKNKTQISQVKLPYAAKLLFQELMSMNIAPRLMVL